European Patent Specification EP 3 760 736 B1, published May 27, 2026. Title: MULTIPLEX TARGET DETECTION ASSAY. Applicant: BRANDEIS UNIVERSITY. The sequence listing filed with the application follows.

SEQUENCE LISTING (103 sequences)

SEQ ID NO: 1 - DNA, 31 bp, Artificial sequence
  Synthetic
ctccagccaggcacgctcacgtgacagaccg

SEQ ID NO: 2 - DNA, 28 bp, Artificial sequence
  Synthetic
acgtggaggcgatcacaccgcagacgtt

SEQ ID NO: 3 - DNA, 37 bp, Artificial sequence
  Synthetic
agcgcccactcgtagccgtacaggatctcgaggaaac

SEQ ID NO: 4 - DNA, 28 bp, Artificial sequence
  Synthetic
tcttgggctggaagagctcgtatggcac

SEQ ID NO: 5 - DNA, 42 bp, Artificial sequence
  Synthetic
ttccggtaaccaggactgaacgggatacgaatgggggtttgg

SEQ ID NO: 6 - DNA, 29 bp, Artificial sequence
  Synthetic
tcgcagccacgttacgctcgtggacatac

SEQ ID NO: 7 - DNA, 37 bp, Artificial sequence
  Synthetic
aactgcccggccagtcgcccgaacgtatggtggacgt

SEQ ID NO: 8 - DNA, 24 bp, Artificial sequence
  Synthetic
gttcatcccggttcggcggtgcca

SEQ ID NO: 9 - DNA, 30 bp, Artificial sequence
  Synthetic
ttcggcgcacaaagtgtctctggctgttgt

SEQ ID NO: 10 - DNA, 27 bp, Artificial sequence
  Synthetic
ggcacgatgctcccacattgcgacttc

SEQ ID NO: 11 - DNA, 16 bp, Artificial sequence
  Synthetic
ctggttggtgcagaag

SEQ ID NO: 12 - DNA, 23 bp, Artificial sequence
  Synthetic
tcaggtccatgaattggctcaga

SEQ ID NO: 13 - DNA, 12 bp, Artificial sequence
  Synthetic
cagcgggttgtt

SEQ ID NO: 14 - DNA, 24 bp, Artificial sequence
  Synthetic
atgcgcttgtggatcaaccccgat

SEQ ID NO: 15 - DNA, 23 bp, Artificial sequence
  Synthetic
aagccccagcgccgacagtcgtt

SEQ ID NO: 16 - DNA, 12 bp, Artificial sequence
  Synthetic
acagaccgccgg

SEQ ID NO: 17 - DNA, 30 bp, Artificial sequence
  Synthetic
actcgcgtccttacccaaaaaaaaaaaaaa

SEQ ID NO: 18 - DNA, 13 bp, Artificial sequence
  Synthetic
atgtcggtggtga

SEQ ID NO: 19 - DNA, 30 bp, Artificial sequence
  Synthetic
aaaaaaaaaaaaaaaggcagtcatcccgtt

SEQ ID NO: 20 - DNA, 19 bp, Artificial sequence
  Synthetic
ttacagcctatcgcctcgc

SEQ ID NO: 21 - DNA, 20 bp, Artificial sequence
  Synthetic
tcggtttgcagctcctgaga

SEQ ID NO: 22 - DNA, 14 bp, Artificial sequence
  Synthetic
gccagcgtcgagtt

SEQ ID NO: 23 - DNA, 35 bp, Artificial sequence
  Synthetic
cgctggaggagatgtgcaccaaaaaaaaaaaaaaa

SEQ ID NO: 24 - DNA, 26 bp, Artificial sequence
  Synthetic
tgtgttggtcgatactaccgtcgccg

SEQ ID NO: 25 - DNA, 22 bp, Artificial sequence
  Synthetic
agggtggacttgacagcgggct

SEQ ID NO: 26 - DNA, 14 bp, Artificial sequence
  Synthetic
gccactagggtgct

SEQ ID NO: 27 - DNA, 18 bp, Artificial sequence
  Synthetic
aatacgcaatggcttgtt

SEQ ID NO: 28 - DNA, 10 bp, Artificial sequence
  Synthetic
gaggacgcgg

SEQ ID NO: 29 - DNA, 23 bp, Artificial sequence
  Synthetic
gtttgtgtgcgctagatggccac

SEQ ID NO: 30 - DNA, 13 bp, Artificial sequence
  Synthetic
ttgccaccgatca

SEQ ID NO: 31 - DNA, 20 bp, Artificial sequence
  Synthetic
tcgtcgatgtggttggtaga

SEQ ID NO: 32 - DNA, 11 bp, Artificial sequence
  Synthetic
gcgtcgatgag

SEQ ID NO: 33 - DNA, 18 bp, Artificial sequence
  Synthetic
atgctgtggcaatgcgat

SEQ ID NO: 34 - DNA, 12 bp, Artificial sequence
  Synthetic
actgctgaattg

SEQ ID NO: 35 - DNA, 25 bp, Artificial sequence
  Synthetic
taagtcgatgagaacggtacgccta

SEQ ID NO: 36 - DNA, 14 bp, Artificial sequence
  Synthetic
agcggcttcgaagg

SEQ ID NO: 37 - DNA, 21 bp, Artificial sequence
  Synthetic
aacctacaccggagcgtactt

SEQ ID NO: 38 - DNA, 14 bp, Artificial sequence
  Synthetic
gttctacaagggtg

SEQ ID NO: 39 - DNA, 35 bp, Artificial sequence
  Synthetic
taggacacgttggcagttgaggcggttaaaaaaaa

SEQ ID NO: 40 - DNA, 22 bp, Artificial sequence
  Synthetic
gcgcggacttctatcccagtct

SEQ ID NO: 41 - DNA, 35 bp, Artificial sequence
  Synthetic
tgtgcgtcagtggtacttccgcaaaaaaaaaaaaa

SEQ ID NO: 42 - DNA, 20 bp, Artificial sequence
  Synthetic
gtgtcgtggctaccgcatac

SEQ ID NO: 43 - DNA, 18 bp, Artificial sequence
  Synthetic
acaccggactattcttcg

SEQ ID NO: 44 - DNA, 22 bp, Artificial sequence
  Synthetic
cccgggtgacgacttctccggc

SEQ ID NO: 45 - DNA, 21 bp, Artificial sequence
  Synthetic
aaccaaggacttccacatcga

SEQ ID NO: 46 - DNA, 34 bp, Artificial sequence
  Synthetic
aacgaagcggtggactatcgttacgttgtggctt

SEQ ID NO: 47 - DNA, 23 bp, Artificial sequence
  Synthetic
cgcgctatcagtgactacctggc

SEQ ID NO: 48 - DNA, 35 bp, Artificial sequence
  Synthetic
ccggtggtgttgtgctggccaaaaaaaaaaaaaaa

SEQ ID NO: 49 - DNA, 25 bp, Artificial sequence
  Synthetic
tgtgagggtggttcgttggcggtaa

SEQ ID NO: 50 - DNA, 27 bp, Artificial sequence
  Synthetic
tttcgttgacgtgcagaacgacttcaa

SEQ ID NO: 51 - DNA, 16 bp, Artificial sequence
  Synthetic
atgcgggcgttgatca

SEQ ID NO: 52 - DNA, 20 bp, Artificial sequence
  Synthetic
attctattatttattttcat

SEQ ID NO: 53 - DNA, 14 bp, Artificial sequence
  Synthetic
atcattatttacta

SEQ ID NO: 54 - DNA, 30 bp, Artificial sequence
  Synthetic
cagctgcactgggaagggtgcagtctgacc

SEQ ID NO: 55 - DNA, 30 bp, Artificial sequence
  Synthetic
ggtcagactgcacccttcccagtgcagctg

SEQ ID NO: 56 - DNA, 22 bp, Artificial sequence
  Synthetic
ggatcagattagcactgatgta

SEQ ID NO: 57 - DNA, 22 bp, Artificial sequence
  Synthetic
tacatcagtgctaatctgatcc

SEQ ID NO: 58 - DNA, 500 bp, Artificial sequence
  Synthetic
cttcacgtaatacaagaaccagcgggggttcggggcacactcaccacgcggggccggtgtggccctaagcgcagtcgagacttgtcgggtagtgcgcctggttctgagcggtgtggagtgggtgcgccctacgtgggggaggcttcacgagcttccgagttgcatctgtgagtgcgagcttaacgagcgagctgctccagtatgtggcatggacacggtccgcgccctcagaatgcgacggcaaaatgctcgcgagctgcggtccgccgtaccgatggtaccagataagagacctgttaggcaacctgttcaacggggcatgctctcaagtggatagactccaccagtgctggaggactcggcatgtctcggaggtcgaggcatggcacgatgctcccctattgcgacttccgggctcgaaggaaccgatgccaaaagcaacagccagagacactttgtgcgccgactgcctaggtctggtcagcaattcccaatacagc

SEQ ID NO: 59 - DNA, 400 bp, Artificial sequence
  Synthetic
cttcacgtaatacaagaagcagcgggttcgggagtgtcacagtgggttgccgtgtgtaagagtcgagacttgtcgggtagtcctggttgtgtggtcgaacgcattagcttgggtcaacgagcttccgagttgcatctgtgagtttaacgagagccagtatgtagcgtcagaatgcagaatcagcaggcacgtgtccgccgtagatggtaccagataagagacctgttaggcaacctgttcaaaatactactctggaggactgagatggcacgatgctcccacattgcgacttctgcccttgatagttatattgaaagtaaatagtagatagtagatgatgatataaacaacagccagagacactttgtgcgccgactgcctatcaaattcccaatacagc

SEQ ID NO: 60 - DNA, 44 bp, Artificial sequence
  Synthetic
gaataatatagccccccccccccccccccccccctatattattc

SEQ ID NO: 61 - DNA, 191 bp, Artificial sequence
  Synthetic
acgtggaggcgatcacaccgcagacgttgatcaacatccggccggtggtcgccgcgatcaaggagttcttcggcaccagccagctgagccaattcatggaccagaacaacccgctgtcggggttgacccacaagcgccgactgtcggcgctggggcccggcggtctgtcacgtgagcgtgccgggctggag

SEQ ID NO: 62 - DNA, 139 bp, Artificial sequence
  Synthetic
gcttgggctggaagagctcgtatggcaccggaaccggtaaggacgcgatcaccagcggcatcgaggtcgtatggacgaacaccccgacgaaatgggacaacagtttcctcgagatcctgtacggctacgagtgggagct

SEQ ID NO: 63 - DNA, 139 bp, Artificial sequence
  Synthetic
tcgcagccacgttacgctcgtggacataccgatttcggcccggccgcggcgagacgataggttgtcggggtgactgccacagccactgaaggggccaaacccccattcgtatcccgttcagtcctggttaccggaggaa

SEQ ID NO: 64 - DNA, 110 bp, Artificial sequence
  Synthetic
ggcacgatgctcccacattgcgacttctgcccttgatagttatattgaaagtaaatagtagatagtagatgatgatataaacaacagccagagacactttgtgcgccgaa

SEQ ID NO: 65 - DNA, 24 bp, Artificial sequence
  Synthetic
aacgccgcgctggaggagatgctt

SEQ ID NO: 66 - DNA, 15 bp, Artificial sequence
  Synthetic
ggccgataccaccgt

SEQ ID NO: 67 - DNA, 24 bp, Artificial sequence
  Synthetic
accatcggagcgtacagcggctgt

SEQ ID NO: 68 - DNA, 15 bp, Artificial sequence
  Synthetic
ctacaagggtgccta

SEQ ID NO: 69 - DNA, 24 bp, Artificial sequence
  Synthetic
acagttggtttgcagctcctgagt

SEQ ID NO: 70 - DNA, 15 bp, Artificial sequence
  Synthetic
gcactgccggcgtcg

SEQ ID NO: 71 - DNA, 24 bp, Artificial sequence
  Synthetic
aagacccgggtgatcacttctctt

SEQ ID NO: 72 - DNA, 15 bp, Artificial sequence
  Synthetic
aaggacttccacatc

SEQ ID NO: 73 - DNA, 24 bp, Artificial sequence
  Synthetic
aacgctatcagtgactacctggtt

SEQ ID NO: 74 - DNA, 15 bp, Artificial sequence
  Synthetic
cgctgcgttggctcg

SEQ ID NO: 75 - DNA, 24 bp, Artificial sequence
  Synthetic
aatcggcaattgagtcggtgtttt

SEQ ID NO: 76 - DNA, 13 bp, Artificial sequence
  Synthetic
cagtctggacgcg

SEQ ID NO: 77 - DNA, 25 bp, Artificial sequence
  Synthetic
tagcggtacgcaatggcttggccta

SEQ ID NO: 78 - DNA, 14 bp, Artificial sequence
  Synthetic
agacggccgaggac

SEQ ID NO: 79 - DNA, 24 bp, Artificial sequence
  Synthetic
acaccatcacgtcgtggcaaccgt

SEQ ID NO: 80 - DNA, 15 bp, Artificial sequence
  Synthetic
ccggagcggcgggct

SEQ ID NO: 81 - DNA, 26 bp, Artificial sequence
  Synthetic
acctctcggcgtggacttctatccgt

SEQ ID NO: 82 - DNA, 15 bp, Artificial sequence
  Synthetic
attgcgttagcggta

SEQ ID NO: 83 - DNA, 24 bp, Artificial sequence
  Synthetic
tttcgttgacgtgcagaatgacaa

SEQ ID NO: 84 - DNA, 15 bp, Artificial sequence
  Synthetic
tgcgggtgttggtca

SEQ ID NO: 85 - DNA, 24 bp, Artificial sequence
  Synthetic
aaagaatggtacgtcactgctgtt

SEQ ID NO: 86 - DNA, 15 bp, Artificial sequence
  Synthetic
tcggaggagttgacg

SEQ ID NO: 87 - DNA, 24 bp, Artificial sequence
  Synthetic
acttcctcgtcgtggccatcgcgt

SEQ ID NO: 88 - DNA, 15 bp, Artificial sequence
  Synthetic
cggcacactggacta

SEQ ID NO: 89 - DNA, 24 bp, Artificial sequence
  Synthetic
agcgcggcgtcgatgaggttgact

SEQ ID NO: 90 - DNA, 15 bp, Artificial sequence
  Synthetic
aattggctgcggtaa

SEQ ID NO: 91 - DNA, 24 bp, Artificial sequence
  Synthetic
aatcgctggcggtaactggtggtt

SEQ ID NO: 92 - DNA, 15 bp, Artificial sequence
  Synthetic
ttctgcgagggtggc

SEQ ID NO: 93 - DNA, 24 bp, Artificial sequence
  Synthetic
aacatcgatcattgtgtgcgcctt

SEQ ID NO: 94 - DNA, 15 bp, Artificial sequence
  Synthetic
tgtggtcggtattgc

SEQ ID NO: 95 - DNA, 24 bp, Artificial sequence
  Synthetic
aagacttgacagcgggtgtgtctt

SEQ ID NO: 96 - DNA, 15 bp, Artificial sequence
  Synthetic
actagggtgctggtg

SEQ ID NO: 97 - DNA, 24 bp, Artificial sequence
  Synthetic
ttccgaacgtatggtggatgtaaa

SEQ ID NO: 98 - DNA, 15 bp, Artificial sequence
  Synthetic
tgcttgggcagttgc

SEQ ID NO: 99 - DNA, 15 bp, Artificial sequence
  Synthetic
aattggctgtggcgg

SEQ ID NO: 100 - DNA, 16 bp, Artificial sequence
  Synthetic
ctggttggtgctgaag

SEQ ID NO: 101 - DNA, 24 bp, Artificial sequence
  Synthetic
atgcgcttgttggtcaaccccgat

SEQ ID NO: 102 - DNA, 23 bp, Artificial sequence
  Synthetic
aagccccagcgccgtcagtcgtt

SEQ ID NO: 103 - DNA, 82 bp, Artificial sequence
  Synthetic
ggcacgatgctcccacattgcgacttccgggctcgaaggaaccgatgccaaaacaacagccagagacactttgtgcgccgaa